European Patent Application EP 4 410 966 A1, published August 7, 2024. Title: CHIMERIC ANTIGEN RECEPTOR IMMUNE CELL, AND PREPARATION METHOD THEREFOR AND APPLICATION THEREOF. Applicant: GRACELL BIOTECHNOLOGIES (SHANGHAI) CO., LTD. The sequence listing filed with the application follows.

SEQUENCE LISTING (24 sequences)

SEQ ID NO: 1 - protein, 395 aa, synthetic construct
  source 1..395: note = Mutant of IL-15/IL-15Ra
MDWTWILFLVAAATRVHSNWVNVISDLKKIEDLIQSMHIDATLYTESDVHPSCKVTAMKCFLLELQVISLESGDASIHDTVENLIILANDSLSSNGNVTESGCKECEELEEKNIKEFLQSFVHIVQMFINTSSGGGSGGGGSGGGGSGGGGSGGGSLQITCPPPMSVEHADIWVKSYSLYSRERYICNSGFKRKAGTSSLTECVLNKATNVAHWTTPSLKCIRDPALVHQRPAPPSTVTTAGVTPQPESLSPSGKEPAASSPSSNNTAATTAAIVPGSQLMPSKSPSTGTTEISSHESSHGTPSQTTAKNWELTASASHQPPGVYPQGHSDTTVAISTSTVLLCGLSAVSLLACYLKSRQTPPLASVEMEAMEALPVTWGTSSRDEDLENCSHHL

SEQ ID NO: 2 - protein, 22 aa, Homo sapiens
MGRGLLRGLWPLHIVLWTRIAS

SEQ ID NO: 3 - protein, 169 aa, Homo sapiens
TIPPHVQKSDVEMEAQKDEIICPSCNRTAHPLRHINNDMIVTDNNGAVKFPQLCKFCDVRFSTCDNQKSCMSNCSITSICEKPQEVCVAVWRKNDENITLETVCHDPKLPYHDFILEDAASPKCIMKEKKKPGETFFMCSCSSDECNDNIIFSEEYNTSNPDLLLVIFQ

SEQ ID NO: 4 - protein, 144 aa, Homo sapiens
TIPPHVQKSVNNDMIVTDNNGAVKFPQLCKFCDVRFSTCDNQKSCMSNCSITSICEKPQEVCVAVWRKNDENITLETVCHDPKLPYHDFILEDAASPKCIMKEKKKPGETFFMCSCSSDECNDNIIFSEEYNTSNPDLLLVIFQ

SEQ ID NO: 5 - protein, 25 aa, Homo sapiens
PILLTISILSFFSVALLVILACVLW

SEQ ID NO: 6 - protein, 28 aa, Homo sapiens
PILLTCPTISILSFFSVALLVILACVLW

SEQ ID NO: 7 - protein, 195 aa, Homo sapiens
KKRIKPIVWPSLPDHKKTLEHLCKKPRKNLNVSFNPESFLDCQIHRVDDIQARDEVEGFLQDTFPQQLEESEKQRLGGDVQSPNCPSEDVVITPESFGRDSSLTCLAGNVSACDAPILSSSRSLDCRESGKNGPHVYQDLLLSLGTTNSTLPPPFSLQSGILTLNPVAQGQPILTSLGSNQEEAYVTMSSFYQNQ

SEQ ID NO: 8 - protein, 933 aa, synthetic construct
  source 1..933: note = Chimeric Antigen Receptor named MesoCAR01
MALPVTALLLPLALLLHAARPQVQLQQSGPGLVTPSQTLSLTCAISGDSVSSNSATWNWIRQSPSRGLEWLGRTYYRSKWYNDYAVSVKSRMSINPDTSKNQFSLQLNSVTPEDTAVYYCARGMMTYYYGMDVWGQGTTVTVSSGILGSGGGGSGGGGSGGGGSQPVLTQSSSLSASPGASASLTCTLRSGINVGPYRIYWYQQKPGSPPQYLLNYKSDSDKQQGSGVPSRFSGSKDASANAGVLLISGLRSEDEADYYCMIWHSSAAVFGGGTQLTVLTTTPAPRPPTPAPTIASQPLSLRPEACRPAAGGAVHTRGLDFACDFWVLVVVGGVLACYSLLVTVAFIIFWVRSKRSRLLHSDYMNMTPRRPGPTRKHYQPYAPPRDFAAYRSRVKFSRSADAPAYQQGQNQLYNELNLGRREEYDVLDKRRGRDPEMGGKPRRKNPQEGLYNELQKDKMAEAYSEIGMKGERRRGKGHDGLYQGLSTATKDTYDALHMQALPPREGRGSLLTCGDVEENPGPMGRGLLRGLWPLHIVLWTRIASTIPPHVQKSDVEMEAQKDEIICPSCNRTAHPLRHINNDMIVTDNNGAVKFPQLCKFCDVRFSTCDNQKSCMSNCSITSICEKPQEVCVAVWRKNDENITLETVCHDPKLPYHDFILEDAASPKCIMKEKKKPGETFFMCSCSSDECNDNIIFSEEYNTSNPDLLLVIFQPILLTISILSFFSVALLVILACVLWKKRIKPIVWPSLPDHKKTLEHLCKKPRKNLNVSFNPESFLDCQIHRVDDIQARDEVEGFLQDTFPQQLEESEKQRLGGDVQSPNCPSEDVVITPESFGRDSSLTCLAGNVSACDAPILSSSRSLDCRESGKNGPHVYQDLLLSLGTTNSTLPPPFSLQSGILTLNPVAQGQPILTSLGSNQEEAYVTMSSFYQNQ

SEQ ID NO: 9 - protein, 908 aa, synthetic construct
  source 1..908: note = Chimeric Antigen Receptor named MesoCAR02
MALPVTALLLPLALLLHAARPQVQLQQSGPGLVTPSQTLSLTCAISGDSVSSNSATWNWIRQSPSRGLEWLGRTYYRSKWYNDYAVSVKSRMSINPDTSKNQFSLQLNSVTPEDTAVYYCARGMMTYYYGMDVWGQGTTVTVSSGILGSGGGGSGGGGSGGGGSQPVLTQSSSLSASPGASASLTCTLRSGINVGPYRIYWYQQKPGSPPQYLLNYKSDSDKQQGSGVPSRFSGSKDASANAGVLLISGLRSEDEADYYCMIWHSSAAVFGGGTQLTVLTTTPAPRPPTPAPTIASQPLSLRPEACRPAAGGAVHTRGLDFACDFWVLVVVGGVLACYSLLVTVAFIIFWVRSKRSRLLHSDYMNMTPRRPGPTRKHYQPYAPPRDFAAYRSRVKFSRSADAPAYQQGQNQLYNELNLGRREEYDVLDKRRGRDPEMGGKPRRKNPQEGLYNELQKDKMAEAYSEIGMKGERRRGKGHDGLYQGLSTATKDTYDALHMQALPPREGRGSLLTCGDVEENPGPMGRGLLRGLWPLHIVLWTRIASTIPPHVQKSVNNDMIVTDNNGAVKFPQLCKFCDVRFSTCDNQKSCMSNCSITSICEKPQEVCVAVWRKNDENITLETVCHDPKLPYHDFILEDAASPKCIMKEKKKPGETFFMCSCSSDECNDNIIFSEEYNTSNPDLLLVIFQPILLTISILSFFSVALLVILACVLWKKRIKPIVWPSLPDHKKTLEHLCKKPRKNLNVSFNPESFLDCQIHRVDDIQARDEVEGFLQDTFPQQLEESEKQRLGGDVQSPNCPSEDVVITPESFGRDSSLTCLAGNVSACDAPILSSSRSLDCRESGKNGPHVYQDLLLSLGTTNSTLPPPFSLQSGILTLNPVAQGQPILTSLGSNQEEAYVTMSSFYQNQ

SEQ ID NO: 10 - protein, 936 aa, synthetic construct
  source 1..936: note = Chimeric Antigen Receptor named MesoCAR03
MALPVTALLLPLALLLHAARPQVQLQQSGPGLVTPSQTLSLTCAISGDSVSSNSATWNWIRQSPSRGLEWLGRTYYRSKWYNDYAVSVKSRMSINPDTSKNQFSLQLNSVTPEDTAVYYCARGMMTYYYGMDVWGQGTTVTVSSGILGSGGGGSGGGGSGGGGSQPVLTQSSSLSASPGASASLTCTLRSGINVGPYRIYWYQQKPGSPPQYLLNYKSDSDKQQGSGVPSRFSGSKDASANAGVLLISGLRSEDEADYYCMIWHSSAAVFGGGTQLTVLTTTPAPRPPTPAPTIASQPLSLRPEACRPAAGGAVHTRGLDFACDFWVLVVVGGVLACYSLLVTVAFIIFWVRSKRSRLLHSDYMNMTPRRPGPTRKHYQPYAPPRDFAAYRSRVKFSRSADAPAYQQGQNQLYNELNLGRREEYDVLDKRRGRDPEMGGKPRRKNPQEGLYNELQKDKMAEAYSEIGMKGERRRGKGHDGLYQGLSTATKDTYDALHMQALPPREGRGSLLTCGDVEENPGPMGRGLLRGLWPLHIVLWTRIASTIPPHVQKSDVEMEAQKDEIICPSCNRTAHPLRHINNDMIVTDNNGAVKFPQLCKFCDVRFSTCDNQKSCMSNCSITSICEKPQEVCVAVWRKNDENITLETVCHDPKLPYHDFILEDAASPKCIMKEKKKPGETFFMCSCSSDECNDNIIFSEEYNTSNPDLLLVIFQPILLTCPTISILSFFSVALLVILACVLWKKRIKPIVWPSLPDHKKTLEHLCKKPRKNLNVSFNPESFLDCQIHRVDDIQARDEVEGFLQDTFPQQLEESEKQRLGGDVQSPNCPSEDVVITPESFGRDSSLTCLAGNVSACDAPILSSSRSLDCRESGKNGPHVYQDLLLSLGTTNSTLPPPFSLQSGILTLNPVAQGQPILTSLGSNQEEAYVTMSSFYQNQ

SEQ ID NO: 11 - protein, 911 aa, synthetic construct
  source 1..911: note = Chimeric Antigen Receptor named MesoCAR04
MALPVTALLLPLALLLHAARPQVQLQQSGPGLVTPSQTLSLTCAISGDSVSSNSATWNWIRQSPSRGLEWLGRTYYRSKWYNDYAVSVKSRMSINPDTSKNQFSLQLNSVTPEDTAVYYCARGMMTYYYGMDVWGQGTTVTVSSGILGSGGGGSGGGGSGGGGSQPVLTQSSSLSASPGASASLTCTLRSGINVGPYRIYWYQQKPGSPPQYLLNYKSDSDKQQGSGVPSRFSGSKDASANAGVLLISGLRSEDEADYYCMIWHSSAAVFGGGTQLTVLTTTPAPRPPTPAPTIASQPLSLRPEACRPAAGGAVHTRGLDFACDFWVLVVVGGVLACYSLLVTVAFIIFWVRSKRSRLLHSDYMNMTPRRPGPTRKHYQPYAPPRDFAAYRSRVKFSRSADAPAYQQGQNQLYNELNLGRREEYDVLDKRRGRDPEMGGKPRRKNPQEGLYNELQKDKMAEAYSEIGMKGERRRGKGHDGLYQGLSTATKDTYDALHMQALPPREGRGSLLTCGDVEENPGPMGRGLLRGLWPLHIVLWTRIASTIPPHVQKSVNNDMIVTDNNGAVKFPQLCKFCDVRFSTCDNQKSCMSNCSITSICEKPQEVCVAVWRKNDENITLETVCHDPKLPYHDFILEDAASPKCIMKEKKKPGETFFMCSCSSDECNDNIIFSEEYNTSNPDLLLVIFQPILLTCPTISILSFFSVALLVILACVLWKKRIKPIVWPSLPDHKKTLEHLCKKPRKNLNVSFNPESFLDCQIHRVDDIQARDEVEGFLQDTFPQQLEESEKQRLGGDVQSPNCPSEDVVITPESFGRDSSLTCLAGNVSACDAPILSSSRSLDCRESGKNGPHVYQDLLLSLGTTNSTLPPPFSLQSGILTLNPVAQGQPILTSLGSNQEEAYVTMSSFYQNQ

SEQ ID NO: 12 - protein, 713 aa, synthetic construct
  source 1..713: note = Chimeric Antigen Receptor named MesoCAR05
MALPVTALLLPLALLLHAARPQVQLQQSGPGLVTPSQTLSLTCAISGDSVSSNSATWNWIRQSPSRGLEWLGRTYYRSKWYNDYAVSVKSRMSINPDTSKNQFSLQLNSVTPEDTAVYYCARGMMTYYYGMDVWGQGTTVTVSSGILGSGGGGSGGGGSGGGGSQPVLTQSSSLSASPGASASLTCTLRSGINVGPYRIYWYQQKPGSPPQYLLNYKSDSDKQQGSGVPSRFSGSKDASANAGVLLISGLRSEDEADYYCMIWHSSAAVFGGGTQLTVLTTTPAPRPPTPAPTIASQPLSLRPEACRPAAGGAVHTRGLDFACDFWVLVVVGGVLACYSLLVTVAFIIFWVRSKRSRLLHSDYMNMTPRRPGPTRKHYQPYAPPRDFAAYRSRVKFSRSADAPAYQQGQNQLYNELNLGRREEYDVLDKRRGRDPEMGGKPRRKNPQEGLYNELQKDKMAEAYSEIGMKGERRRGKGHDGLYQGLSTATKDTYDALHMQALPPREGRGSLLTCGDVEENPGPMGRGLLRGLWPLHIVLWTRIASTIPPHVQKSDVEMEAQKDEIICPSCNRTAHPLRHINNDMIVTDNNGAVKFPQLCKFCDVRFSTCDNQKSCMSNCSITSICEKPQEVCVAVWRKNDENITLETVCHDPKLPYHDFILEDAASPKCIMKEKKKPGETFFMCSCSSDECNDNIIFSEEYNTSNPDLLLVIFQ

SEQ ID NO: 13 - protein, 688 aa, synthetic construct
  source 1..688: note = Chimeric Antigen Receptor named MesoCAR06
MALPVTALLLPLALLLHAARPQVQLQQSGPGLVTPSQTLSLTCAISGDSVSSNSATWNWIRQSPSRGLEWLGRTYYRSKWYNDYAVSVKSRMSINPDTSKNQFSLQLNSVTPEDTAVYYCARGMMTYYYGMDVWGQGTTVTVSSGILGSGGGGSGGGGSGGGGSQPVLTQSSSLSASPGASASLTCTLRSGINVGPYRIYWYQQKPGSPPQYLLNYKSDSDKQQGSGVPSRFSGSKDASANAGVLLISGLRSEDEADYYCMIWHSSAAVFGGGTQLTVLTTTPAPRPPTPAPTIASQPLSLRPEACRPAAGGAVHTRGLDFACDFWVLVVVGGVLACYSLLVTVAFIIFWVRSKRSRLLHSDYMNMTPRRPGPTRKHYQPYAPPRDFAAYRSRVKFSRSADAPAYQQGQNQLYNELNLGRREEYDVLDKRRGRDPEMGGKPRRKNPQEGLYNELQKDKMAEAYSEIGMKGERRRGKGHDGLYQGLSTATKDTYDALHMQALPPREGRGSLLTCGDVEENPGPMGRGLLRGLWPLHIVLWTRIASTIPPHVQKSVNNDMIVTDNNGAVKFPQLCKFCDVRFSTCDNQKSCMSNCSITSICEKPQEVCVAVWRKNDENITLETVCHDPKLPYHDFILEDAASPKCIMKEKKKPGETFFMCSCSSDECNDNIIFSEEYNTSNPDLLLVIFQ

SEQ ID NO: 14 - protein, 1127 aa, synthetic construct
  source 1..1127: note = Chimeric Antigen Receptor named MesoCAR07
MALPVTALLLPLALLLHAARPQVQLQQSGPGLVTPSQTLSLTCAISGDSVSSNSATWNWIRQSPSRGLEWLGRTYYRSKWYNDYAVSVKSRMSINPDTSKNQFSLQLNSVTPEDTAVYYCARGMMTYYYGMDVWGQGTTVTVSSGILGSGGGGSGGGGSGGGGSQPVLTQSSSLSASPGASASLTCTLRSGINVGPYRIYWYQQKPGSPPQYLLNYKSDSDKQQGSGVPSRFSGSKDASANAGVLLISGLRSEDEADYYCMIWHSSAAVFGGGTQLTVLTTTPAPRPPTPAPTIASQPLSLRPEACRPAAGGAVHTRGLDFACDFWVLVVVGGVLACYSLLVTVAFIIFWVRSKRSRLLHSDYMNMTPRRPGPTRKHYQPYAPPRDFAAYRSRVKFSRSADAPAYQQGQNQLYNELNLGRREEYDVLDKRRGRDPEMGGKPRRKNPQEGLYNELQKDKMAEAYSEIGMKGERRRGKGHDGLYQGLSTATKDTYDALHMQALPPRATNFSLLKQAGDVEENPGPMDWTWILFLVAAATRVHSNWVNVISDLKKIEDLIQSMHIDATLYTESDVHPSCKVTAMKCFLLELQVISLESGDASIHDTVENLIILANDSLSSNGNVTESGCKECEELEEKNIKEFLQSFVHIVQMFINTSSGGGSGGGGSGGGGSGGGGSGGGSLQITCPPPMSVEHADIWVKSYSLYSRERYICNSGFKRKAGTSSLTECVLNKATNVAHWTTPSLKCIRDPALVHQRPAPPSTVTTAGVTPQPESLSPSGKEPAASSPSSNNTAATTAAIVPGSQLMPSKSPSTGTTEISSHESSHGTPSQTTAKNWELTASASHQPPGVYPQGHSDTTVAISTSTVLLCGLSAVSLLACYLKSRQTPPLASVEMEAMEALPVTWGTSSRDEDLENCSHHLEGRGSLLTCGDVEENPGPMGRGLLRGLWPLHIVLWTRIASTIPPHVQKSDVEMEAQKDEIICPSCNRTAHPLRHINNDMIVTDNNGAVKFPQLCKFCDVRFSTCDNQKSCMSNCSITSICEKPQEVCVAVWRKNDENITLETVCHDPKLPYHDFILEDAASPKCIMKEKKKPGETFFMCSCSSDECNDNIIFSEEYNTSNPDLLLVIFQ

SEQ ID NO: 15 - protein, 1101 aa, synthetic construct
  source 1..1101: note = Chimeric Antigen Receptor named MesoCAR08
MALPVTALLLPLALLLHAARPQVQLQQSGPGLVTPSQTLSLTCAISGDSVSSNSATWNWIRQSPSRGLEWLGRTYYRSKWYNDYAVSVKSRMSINPDTSKNQFSLQLNSVTPEDTAVYYCARGMMTYYYGMDVWGQGTTVTVSSGILGSGGGGSGGGGSGGGGSQPVLTQSSSLSASPGASASLTCTLRSGINVGPYRIYWYQQKPGSPPQYLLNYKSDSDKQQGSGVPSRFSGSKDASANAGVLLISGLRSEDEADYYCMIWHSSAAVFGGGTQLTVLTTTPAPRPPTPAPTIASQPLSLRPEACRPAAGGAVHTRGLDFACDFWVLVVVGGVLACYSLLVTVAFIIFWVRSKRSRLLHSDYMNMTPRRPGPTRKHYQPYAPPRDFAAYRSRVKFSRSADAPAYQQGQNQLYNELNLGRREEYDVLDKRRGRDPEMGGKPRRKNPQEGLYNELQKDKMAEAYSEIGMKGERRRGKGHDGLYQGLSTATKDTYDALHMQALPPRATNFSLLKQAGDVEENPGPMDWTWILFLVAAATRVHSNWVNVISDLKKIEDLIQSMHIDATLYTESDVHPSCKVTAMKCFLLELQVISLESGDASIHDTVENLIILANDSLSSNGNVTESGCKECEELEEKNIKEFLQSFVHIVQMFINTSSGGGSGGGGSGGGGSGGGGSGGGSLQITCPPPMSVEHADIWVKSYSLYSRERYICNSGFKRKAGTSSLTECVLNKATNVAHWTTPSLKCIRDPALVHQRPAPPSTVTTAGVTPQPESLSPSGKEPAASSPSSNNTAATTAAIVPGSQLMPSKSPSTGTTEISSHESSHGTPSQTTAKNWELTASASHQPPGVYPQGHSDTTVAISTSTVLLCGLSAVSLLACYLKSRQTPPLASVEMEAMEALPVTWGTSSRDEDLENCSHHLEGRGSLLTCGDVEENPGPGRGLLRGLWPLHIVLWTRIASTIPPHVQKSVNNDMIVTDNNGAVKFPQLCKFCDVRFSTCDNQKSCMSNCSITSICEKPQEVCVAVWRKNDENITLETVCHDPKLPYHDFILEDAASPKCIMKEKKKPGETFFMCSCSSDECNDNIIFSEEYNTSNPDLLLVIFQ

SEQ ID NO: 16 - protein, 1347 aa, synthetic construct
  source 1..1347: note = Chimeric Antigen Receptor named MesoCAR09
MALPVTALLLPLALLLHAARPQVQLQQSGPGLVTPSQTLSLTCAISGDSVSSNSATWNWIRQSPSRGLEWLGRTYYRSKWYNDYAVSVKSRMSINPDTSKNQFSLQLNSVTPEDTAVYYCARGMMTYYYGMDVWGQGTTVTVSSGILGSGGGGSGGGGSGGGGSQPVLTQSSSLSASPGASASLTCTLRSGINVGPYRIYWYQQKPGSPPQYLLNYKSDSDKQQGSGVPSRFSGSKDASANAGVLLISGLRSEDEADYYCMIWHSSAAVFGGGTQLTVLTTTPAPRPPTPAPTIASQPLSLRPEACRPAAGGAVHTRGLDFACDFWVLVVVGGVLACYSLLVTVAFIIFWVRSKRSRLLHSDYMNMTPRRPGPTRKHYQPYAPPRDFAAYRSRVKFSRSADAPAYQQGQNQLYNELNLGRREEYDVLDKRRGRDPEMGGKPRRKNPQEGLYNELQKDKMAEAYSEIGMKGERRRGKGHDGLYQGLSTATKDTYDALHMQALPPRATNFSLLKQAGDVEENPGPMDWTWILFLVAAATRVHSNWVNVISDLKKIEDLIQSMHIDATLYTESDVHPSCKVTAMKCFLLELQVISLESGDASIHDTVENLIILANDSLSSNGNVTESGCKECEELEEKNIKEFLQSFVHIVQMFINTSSGGGSGGGGSGGGGSGGGGSGGGSLQITCPPPMSVEHADIWVKSYSLYSRERYICNSGFKRKAGTSSLTECVLNKATNVAHWTTPSLKCIRDPALVHQRPAPPSTVTTAGVTPQPESLSPSGKEPAASSPSSNNTAATTAAIVPGSQLMPSKSPSTGTTEISSHESSHGTPSQTTAKNWELTASASHQPPGVYPQGHSDTTVAISTSTVLLCGLSAVSLLACYLKSRQTPPLASVEMEAMEALPVTWGTSSRDEDLENCSHHLEGRGSLLTCGDVEENPGPMGRGLLRGLWPLHIVLWTRIASTIPPHVQKSDVEMEAQKDEIICPSCNRTAHPLRHINNDMIVTDNNGAVKFPQLCKFCDVRFSTCDNQKSCMSNCSITSICEKPQEVCVAVWRKNDENITLETVCHDPKLPYHDFILEDAASPKCIMKEKKKPGETFFMCSCSSDECNDNIIFSEEYNTSNPDLLLVIFQPILLTISILSFFSVALLVILACVLWKKRIKPIVWPSLPDHKKTLEHLCKKPRKNLNVSFNPESFLDCQIHRVDDIQARDEVEGFLQDTFPQQLEESEKQRLGGDVQSPNCPSEDVVITPESFGRDSSLTCLAGNVSACDAPILSSSRSLDCRESGKNGPHVYQDLLLSLGTTNSTLPPPFSLQSGILTLNPVAQGQPILTSLGSNQEEAYVTMSSFYQNQ

SEQ ID NO: 17 - protein, 1350 aa, synthetic construct
  source 1..1350: note = Chimeric Antigen Receptor named MesoCAR10
MALPVTALLLPLALLLHAARPQVQLQQSGPGLVTPSQTLSLTCAISGDSVSSNSATWNWIRQSPSRGLEWLGRTYYRSKWYNDYAVSVKSRMSINPDTSKNQFSLQLNSVTPEDTAVYYCARGMMTYYYGMDVWGQGTTVTVSSGILGSGGGGSGGGGSGGGGSQPVLTQSSSLSASPGASASLTCTLRSGINVGPYRIYWYQQKPGSPPQYLLNYKSDSDKQQGSGVPSRFSGSKDASANAGVLLISGLRSEDEADYYCMIWHSSAAVFGGGTQLTVLTTTPAPRPPTPAPTIASQPLSLRPEACRPAAGGAVHTRGLDFACDFWVLVVVGGVLACYSLLVTVAFIIFWVRSKRSRLLHSDYMNMTPRRPGPTRKHYQPYAPPRDFAAYRSRVKFSRSADAPAYQQGQNQLYNELNLGRREEYDVLDKRRGRDPEMGGKPRRKNPQEGLYNELQKDKMAEAYSEIGMKGERRRGKGHDGLYQGLSTATKDTYDALHMQALPPRATNFSLLKQAGDVEENPGPMDWTWILFLVAAATRVHSNWVNVISDLKKIEDLIQSMHIDATLYTESDVHPSCKVTAMKCFLLELQVISLESGDASIHDTVENLIILANDSLSSNGNVTESGCKECEELEEKNIKEFLQSFVHIVQMFINTSSGGGSGGGGSGGGGSGGGGSGGGSLQITCPPPMSVEHADIWVKSYSLYSRERYICNSGFKRKAGTSSLTECVLNKATNVAHWTTPSLKCIRDPALVHQRPAPPSTVTTAGVTPQPESLSPSGKEPAASSPSSNNTAATTAAIVPGSQLMPSKSPSTGTTEISSHESSHGTPSQTTAKNWELTASASHQPPGVYPQGHSDTTVAISTSTVLLCGLSAVSLLACYLKSRQTPPLASVEMEAMEALPVTWGTSSRDEDLENCSHHLEGRGSLLTCGDVEENPGPMGRGLLRGLWPLHIVLWTRIASTIPPHVQKSDVEMEAQKDEIICPSCNRTAHPLRHINNDMIVTDNNGAVKFPQLCKFCDVRFSTCDNQKSCMSNCSITSICEKPQEVCVAVWRKNDENITLETVCHDPKLPYHDFILEDAASPKCIMKEKKKPGETFFMCSCSSDECNDNIIFSEEYNTSNPDLLLVIFQPILLTCPTISILSFFSVALLVILACVLWKKRIKPIVWPSLPDHKKTLEHLCKKPRKNLNVSFNPESFLDCQIHRVDDIQARDEVEGFLQDTFPQQLEESEKQRLGGDVQSPNCPSEDVVITPESFGRDSSLTCLAGNVSACDAPILSSSRSLDCRESGKNGPHVYQDLLLSLGTTNSTLPPPFSLQSGILTLNPVAQGQPILTSLGSNQEEAYVTMSSFYQNQ

SEQ ID NO: 18 - protein, 921 aa, synthetic construct
  source 1..921: note = Chimeric Antigen Receptor named E1m1
MALPVTALLLPLALLLHAARPQVQLQQSGPGLVTPSQTLSLTCAISGDSVSSNSATWNWIRQSPSRGLEWLGRTYYRSKWYNDYAVSVKSRMSINPDTSKNQFSLQLNSVTPEDTAVYYCARGMMTYYYGMDVWGQGTTVTVSSGILGSGGGGSGGGGSGGGGSQPVLTQSSSLSASPGASASLTCTLRSGINVGPYRIYWYQQKPGSPPQYLLNYKSDSDKQQGSGVPSRFSGSKDASANAGVLLISGLRSEDEADYYCMIWHSSAAVFGGGTQLTVLTTTPAPRPPTPAPTIASQPLSLRPEACRPAAGGAVHTRGLDFACDFWVLVVVGGVLACYSLLVTVAFIIFWVRSKRSRLLHSDYMNMTPRRPGPTRKHYQPYAPPRDFAAYRSRVKFSRSADAPAYQQGQNQLYNELNLGRREEYDVLDKRRGRDPEMGGKPRRKNPQEGLYNELQKDKMAEAYSEIGMKGERRRGKGHDGLYQGLSTATKDTYDALHMQALPPRGSGATNFSLLKQAGDVEENPGPMDWTWILFLVAAATRVHSNWVNVISDLKKIEDLIQSMHIDATLYTESDVHPSCKVTAMKCFLLELQVISLESGDASIHDTVENLIILANDSLSSNGNVTESGCKECEELEEKNIKEFLQSFVHIVQMFINTSSGGGSGGGGSGGGGSGGGGSGGGSLQITCPPPMSVEHADIWVKSYSLYSRERYICNSGFKRKAGTSSLTECVLNKATNVAHWTTPSLKCIRDPALVHQRPAPPSTVTTAGVTPQPESLSPSGKEPAASSPSSNNTAATTAAIVPGSQLMPSKSPSTGTTEISSHESSHGTPSQTTAKNWELTASASHQPPGVYPQGHSDTTVAISTSTVLLCGLSAVSLLACYLKSRQTPPLASVEMEAMEALPVTWGTSSRDEDLENCSHHL

SEQ ID NO: 19 - protein, 423 aa, synthetic construct
  source 1..423: note = Amino acid sequence of CAR11
MGRGLLRGLWPLHIVLWTRIASTIPPHVQKSDVEMEAQKDEIICPSCNRTAHPLRHINNDMIVTDNNGAVKFPQLCKFCDVRFSTCDNQKSCMSNCSITSICEKPQEVCVAVWRKNDENITLETVCHDPKLPYHDFILEDAASPKCIMKEKKKPGETFFMCSCSSDECNDNIIFSEECKPDHGYWSAWSPATFIQIPSDFTMNDTTVWISVAVLSAVICLIIVWAVALKKRIKPIVWPSLPDHKKTLEHLCKKPRKNLNVSFNPESFLDCQIHRVDDIQARDEVEGFLQDTFPQQLEESEKQRLGGDVQSPNCPSEDVVITPESFGRDSSLTCLAGNVSACDAPILSSSRSLDCRESGKNGPHVYQDLLLSLGTTNSTLPPPFSLQSGILTLNPVAQGQPILTSLGSNQEEAYVTMSSFYQNQ

SEQ ID NO: 20 - protein, 433 aa, synthetic construct
  source 1..433: note = Amino acid sequence of CAR12
MGRGLLRGLWPLHIVLWTRIASTIPPHVQKSDVEMEAQKDEIICPSCNRTAHPLRHINNDMIVTDNNGAVKFPQLCKFCDVRFSTCDNQKSCMSNCSITSICEKPQEVCVAVWRKNDENITLETVCHDPKLPYHDFILEDAASPKCIMKEKKKPGETFFMCSCSSDECNDNIIFSEEKVRSIPDHYFKGFWSEWSPSYYFRTPEINNSSGEMDPILLTISILSFFSVALLVILACVLWKKRIKPIVWPSLPDHKKTLEHLCKKPRKNLNVSFNPESFLDCQIHRVDDIQARDEVEGFLQDTFPQQLEESEKQRLGGDVQSPNCPSEDVVITPESFGRDSSLTCLAGNVSACDAPILSSSRSLDCRESGKNGPHVYQDLLLSLGTTNSTLPPPFSLQSGILTLNPVAQGQPILTSLGSNQEEAYVTMSSFYQNQ

SEQ ID NO: 21 - protein, 424 aa, synthetic construct
  source 1..424: note = Amino acid sequence of CAR13
MALPVTALLLPLALLLHAARPQLCKFCDVRFSTCDNQKSCMSNCSITSICEKPQEVCVAVWRKNDENITLETVCHDPKLPYHDFILEDAASPKCIMKEKKKPGETFFMCSCSSDECNDNIIFSEEYNTSNPDLLLVIFQSDHLVLGLSAVLGLLLLRWQFPAHYRRLRHALWPSLPDLHRVLGQYLRDTAALSPPKATVSDTCEEVEPSLLEILPKSSERTPLPLLEARDEVEGFLQDTFPQQLEESEKQRLGGDVQSPNCPSEDVVITPESFGRDSSLTCLAGNVSACDAPILSSSRSLDCRESGKNGPHVYQDLLLSLGTTNSTLPPPFSLQSGILTLNPVAQGQPILTSLGSNQEEAYVTMSSFYQNQSRSDPKPENPACPWTVLPAGDLPTHDGYLPSNIDDLPSHEAPLADSLEELEPQ

SEQ ID NO: 22 - protein, 51 aa, Homo sapiens
CKPDHGYWSAWSPATFIQIPSDFTMNDTTVWISVAVLSAVICLIIVWAVAL

SEQ ID NO: 23 - protein, 61 aa, Homo sapiens
KVRSIPDHYFKGFWSEWSPSYYFRTPEINNSSGEMDPILLTISILSFFSVALLVILACVLW

SEQ ID NO: 24 - protein, 17 aa, Homo sapiens
SDHLVLGLSAVLGLLLL